European Patent Application EP 4 574 207 A2, published June 25, 2025. Title: Means and methods for treating copper-related diseases. Applicant: Helmholtz Zentrum Muenchen Deutsches Forschungszentrum fuer Gesundheit und Umwelt (GmbH) et al. Application EP. The sequence listing filed with the application follows.

SEQUENCE LISTING (17 sequences)

SEQ ID NO: 1 - protein, 30 aa, Methylosinus sp.
MTVKIAQKKVLPVIGRAAALCGSCYPCSCM

SEQ ID NO: 2 - protein, 34 aa, Methylosinus sp.
MAIKIAKKEVLPVVGRLGAMCSSCPMCHCGPLCP

SEQ ID NO: 3 - protein, 32 aa, Methylocystis sp.
MAIKISKKEVLPVVGRLGAMCSSCPMCGPLCP

SEQ ID NO: 4 - protein, 32 aa, Methylosinus sp.
MAIKIAKKEVLPVVGRLGAMCSSCPMCGPLCP

SEQ ID NO: 5 - protein, 31 aa, Methylosinus sp.
MTIKVVKKEILPVIGRVQAMCACNPPWCGTC

SEQ ID NO: 6 - protein, 35 aa, Methylocystis sp.
MAIKIVKKEILPVIGRVQAFCSSDSGGGQIGCGPA

SEQ ID NO: 7 - protein, 30 aa, Methylocystis sp.
MTIRIAKRITLNVIGRASARCASTCAATNG

SEQ ID NO: 8 - protein, 30 aa, Methylocystis sp.; identical to SEQ ID NO: 7

SEQ ID NO: 9 - protein, 30 aa, Methylocystis sp.
MTIRIAKRITLNVIGRASAMCASTCAATNG

SEQ ID NO: 10 - protein, 27 aa, Methylocystis sp.
MTIKIVKRTALAVNGRAGADCGTACWA

SEQ ID NO: 11 - protein, 27 aa, Methylocystis sp.
MAINIVKRTTLVVNGRTGADCGTACWG

SEQ ID NO: 12 - protein, 27 aa, Methylosinus sp.
MAINIVKRTTLVVNGRSGADCGTACWG

SEQ ID NO: 13 - protein, 29 aa, Tistrella mobilis
MSIKISARKALQIAGRAGARCATICAVAG

SEQ ID NO: 14 - protein, 30 aa, Cupriavidus basiliensis
MTIKISKKEAIEVRGRSGACCGSCCAAIGA

SEQ ID NO: 15 - protein, 31 aa, Pseudomonas extremaustralis
MSIKIAKKHTLQIAGRAGACCASCCAPLGVN

SEQ ID NO: 16 - protein, 31 aa, Azospirillum sp.
MTIKIAKKQTLSVAGRAGACCGSCCAPVGVN

SEQ ID NO: 17 - protein, 31 aa, Comamonas composti
MKIKVTKKTTMTVAGRAGACCASCCAPVGVN